European Patent Application EP 4 397 312 A1, published July 10, 2024. Title: Therapeutic agent for arthropathy and method for producing therapeutic agent for arthropathy. Applicant: FUJIFILM Corporation. The sequence listing filed with the application follows.

SEQUENCE LISTING (12 sequences)

SEQ ID NO: 1 - DNA, 4538 bp, Rattus norvegicus
  source 1..4538: mol_type = genomic DNA
ggctgccgggtctcctgcctcctcctcctgctcctagagcctcctgcatgagggcgcggtagagacccggacccgctccgtgctctgccgcctcgccgagcttcgcccgggccaaggctctgccaggcctcgcggtgagccatgatccgcctcggggctccccagtcgctggtgctgctgacgctgctcatcgccacggtcctacaatgtcagggccaggatgcccgaaaattagggccaaaggggcagaaaggagaacctggagatatcaaagatatcataggacctaaaggacctcctggccctcagggacctgccggtgaacaaggacccagaggtgaccgtggtgacaagggagagaggggtgcacctggaccccgtggcagagatggagaacctggtacccctggaaatcctggtccccctggccctccaggcccccctggtccccctggccttggtggaggaaactttgcagcccagatggctggaggatttgacgagaaggctggtggtgcccagatgggagtcatgcaaggccccatgggccccatgggacctcgtggacccccaggccccgccggtgcccccggccctcaaggatttcaaggcaatcctggtgaacctggcgagcctggtgtctctggtcccattggtccccgaggtcctccaggtcctgctggaaaacctggtgatgatggtgaagctggaaagcccggaaaggccggagaaagaggcctccctggtcctcagggtgctcgtggattcccgggaacccccggtcttcctggtgtcaagggtcacagaggttacccaggcctcgatggtgctaagggagaagctggtgctccaggtgtgaagggtgagagcggttcccctggtgagaacggatccccaggcccaatgggtccccgtggcctgcctggcgagagaggacggactggccctgctggtgctgctggtgctcgaggcaacgacggccagccaggccctgctggacctccgggtcctgttggtcctgcaggtggtcctggcttccttggtgctcctggtgccaagggcgaagctggtcccactggtgcccgtggtcctgaaggtgctcaaggttctcgtggcgaacccggcaatcccggatcccccgggcccgcaggcgcttctggtaacccagggactgatggtattcccggagccaaaggatctgctggcgctcctggaattgctggtgcccctggcttccctgggccccgtggccctcccggtcctcaaggtgcaactggtcctctgggccccaaaggtcagacgggtgagcccggcatcgctggcttcaaaggtgaacaaggccccaagggagagactggacctgctgggccccagggagcccctggccctgctggtgaagaaggaaaacgaggtgctcgaggagagcccggtggcgctggacctatcggcccccctggagagagaggtgctcctggcaaccgcggtttcccaggtcaagatggtctggcaggtcccaagggtgcccctggagagcgagggcctagtggcctggctggtcctaagggtgccaatggtgacccgggtcgtcctggagaacctggtcttcctggagccaggggtcttactggccgccctggtgatgctggtcctcaaggcaaagttggtccttctggagcccctggagaagacggtcgccctggtcctcctggtcctcagggagctcgtgggcagcctggcgtcatgggtttccctggccccaaaggagccaatggcgagcctggcaaagctggtgagaaaggactggctggtgctcctggtctgagaggtcttcctggcaaagatggtgagacaggagccgcaggaccccccggccccagcggacctgctggtgaacgaggcgagcagggtgctcctgggccatcagggttccagggacttcctggccctcctggtcccccgggtgaaggtggaaagcaaggtgaccagggtattcctggtgaagctggagcccctggcctcgttggtccccggggtgaacgaggtttcccaggtgaacgtggctctcccggtgctcagggcctccagggtccccgaggcctccctggcactcctggtactgatggtcccaaaggtgcggctggcccagatggtccccctggggctcagggccctccaggtctacagggaatgcctggtgagaggggagcagctggtattgctggacccaagggagacagaggtgatgttggcgagaaaggcccagagggagctcctggaaaagatggtggccgaggtcttactgggcccatcgggcccccaggaccagcaggtgccaatggcgagaagggagaagtcggacctcctggtccttcaggaagtactggagctcgaggcgccccgggtgagcgcggagagactgggccacctggacctgctggattcgctggccctcctggtgctgatggccagcctggtgccaagggcgatcaaggagaagctggacagaaaggtgacgctggtgcccctggcccacaaggcccctcaggagctcccgggccacagggtcctactggagtgactggtcctaagggagcccggggcgcccaaggcccaccgggagccaccggattccctggagctgctggccgagttggacccccaggttctaatggcaaccctgggcccgccggtccccctggtcctgctggaaaagatggtcccaaaggtgctcgaggagacactggtgcccctggcagagctggtgaccctggacttcaaggacccgcaggagctcctggagagaaaggcgaacctggagatgacggtccctctggttctgatggtcccccaggtccccaggggctggctggtcaaaggggcattgttggtctgcctggtcagcgtggtgagagaggattcccaggccttcccggcccatcgggtgagcccggcaagcagggtgcacctggtgcatctggagacagaggtcctcctggtcctgtggggcctcctggcttgacaggacctgcaggtgaacctggacgagagggcagccctggtgctgatggaccccctggcagagatggtgcggctggagtcaagggtgatcgtggtgagactggtgcacttggtgctcctggagctcctgggcccccaggctctcctggtcctgctggcccaactggcaaacaaggagacagaggagaggctggtgcacaaggtcctatgggcccctcaggacctgctggagcccgtggaattgctggccctcaaggcccccgaggtgacaaaggagaagctggagagcctggcgagagaggactgaaggggcaccgaggtttcactggactgcagggtctgcctggccccccgggtccttctggagatcagggtacttctggccctgctggtccttccggccctagaggtccacctggccctgttggtccctctggcaaagatggctctaatggaatccctggccccatcgggcctccaggtccccgtggacgctcaggagaaactggccctgctggtcctcctggaaatcctggtccccctggccctccgggtcctcctggtcctggcatcgacatgtcagcctttgctggcttaggacagagagagaagggccccgatcccctgcagtacatgcgggccgacgaggcagacagtaccttgagacagcatgacgtcgaggtggacgccacgctcaagtcgctgaacaaccagatcgagagcatccgcagccctgatggctcccgcaagaatcccgctcgcacctgccaggacctgaaactctgccacccagagtggaagagcggagactactggattgatcccaaccagggctgcaccttggacgccatgaaagtcttctgcaacatggagactggcgagtcttgcgtctaccccaacccagcgactgtgcctcggaagaactggtggagcagcaagagcaaggagaagaagcacatctggtttggagagaccatgaacggcggcttccacttcagctacggcgacggcaacctggctcccaacaccgctaacgtccagatgactttcctccgtctactgtccactgagggctcccagaacatcacctaccactgtaagaacagcattgcctacctggacgaagcagccggcaacctcaagaaggccttgctcatccagggctccaatgatgtggagatgagggccgagggcaacagcaggttcacgtacactgccctgaaggatggctgcacgaaacacaccggtaagtggggcaagaccatcatcgagtaccgatcacagaagacctcacgccttcccattgttgacattgcacccatggacatcggagggcctgatcaggaatttggtgtggacatagggcctgtctgtttcttgtaaaaccctcaaccccaaaacaacacaatccattgcgaacccaaaggacccaaatactttctaaccgcagtcactctaggatctgcactgaatggctgacctgacctgatattcaactatcctaacctcacagtccggac

SEQ ID NO: 2 - DNA, 4539 bp, Rattus norvegicus
  misc_feature 200: note = n is insertion sequence of Col2A1KO-rSMSC
  source 1..4539: mol_type = genomic DNA
ggctgccgggtctcctgcctcctcctcctgctcctagagcctcctgcatgagggcgcggtagagacccggacccgctccgtgctctgccgcctcgccgagcttcgcccgggccaaggctctgccaggcctcgcggtgagccatgatccgcctcggggctccccagtcgctggtgctgctgacgctgctcatcgccacggntcctacaatgtcagggccaggatgcccgaaaattagggccaaaggggcagaaaggagaacctggagatatcaaagatatcataggacctaaaggacctcctggccctcagggacctgccggtgaacaaggacccagaggtgaccgtggtgacaagggagagaggggtgcacctggaccccgtggcagagatggagaacctggtacccctggaaatcctggtccccctggccctccaggcccccctggtccccctggccttggtggaggaaactttgcagcccagatggctggaggatttgacgagaaggctggtggtgcccagatgggagtcatgcaaggccccatgggccccatgggacctcgtggacccccaggccccgccggtgcccccggccctcaaggatttcaaggcaatcctggtgaacctggcgagcctggtgtctctggtcccattggtccccgaggtcctccaggtcctgctggaaaacctggtgatgatggtgaagctggaaagcccggaaaggccggagaaagaggcctccctggtcctcagggtgctcgtggattcccgggaacccccggtcttcctggtgtcaagggtcacagaggttacccaggcctcgatggtgctaagggagaagctggtgctccaggtgtgaagggtgagagcggttcccctggtgagaacggatccccaggcccaatgggtccccgtggcctgcctggcgagagaggacggactggccctgctggtgctgctggtgctcgaggcaacgacggccagccaggccctgctggacctccgggtcctgttggtcctgcaggtggtcctggcttccttggtgctcctggtgccaagggcgaagctggtcccactggtgcccgtggtcctgaaggtgctcaaggttctcgtggcgaacccggcaatcccggatcccccgggcccgcaggcgcttctggtaacccagggactgatggtattcccggagccaaaggatctgctggcgctcctggaattgctggtgcccctggcttccctgggccccgtggccctcccggtcctcaaggtgcaactggtcctctgggccccaaaggtcagacgggtgagcccggcatcgctggcttcaaaggtgaacaaggccccaagggagagactggacctgctgggccccagggagcccctggccctgctggtgaagaaggaaaacgaggtgctcgaggagagcccggtggcgctggacctatcggcccccctggagagagaggtgctcctggcaaccgcggtttcccaggtcaagatggtctggcaggtcccaagggtgcccctggagagcgagggcctagtggcctggctggtcctaagggtgccaatggtgacccgggtcgtcctggagaacctggtcttcctggagccaggggtcttactggccgccctggtgatgctggtcctcaaggcaaagttggtccttctggagcccctggagaagacggtcgccctggtcctcctggtcctcagggagctcgtgggcagcctggcgtcatgggtttccctggccccaaaggagccaatggcgagcctggcaaagctggtgagaaaggactggctggtgctcctggtctgagaggtcttcctggcaaagatggtgagacaggagccgcaggaccccccggccccagcggacctgctggtgaacgaggcgagcagggtgctcctgggccatcagggttccagggacttcctggccctcctggtcccccgggtgaaggtggaaagcaaggtgaccagggtattcctggtgaagctggagcccctggcctcgttggtccccggggtgaacgaggtttcccaggtgaacgtggctctcccggtgctcagggcctccagggtccccgaggcctccctggcactcctggtactgatggtcccaaaggtgcggctggcccagatggtccccctggggctcagggccctccaggtctacagggaatgcctggtgagaggggagcagctggtattgctggacccaagggagacagaggtgatgttggcgagaaaggcccagagggagctcctggaaaagatggtggccgaggtcttactgggcccatcgggcccccaggaccagcaggtgccaatggcgagaagggagaagtcggacctcctggtccttcaggaagtactggagctcgaggcgccccgggtgagcgcggagagactgggccacctggacctgctggattcgctggccctcctggtgctgatggccagcctggtgccaagggcgatcaaggagaagctggacagaaaggtgacgctggtgcccctggcccacaaggcccctcaggagctcccgggccacagggtcctactggagtgactggtcctaagggagcccggggcgcccaaggcccaccgggagccaccggattccctggagctgctggccgagttggacccccaggttctaatggcaaccctgggcccgccggtccccctggtcctgctggaaaagatggtcccaaaggtgctcgaggagacactggtgcccctggcagagctggtgaccctggacttcaaggacccgcaggagctcctggagagaaaggcgaacctggagatgacggtccctctggttctgatggtcccccaggtccccaggggctggctggtcaaaggggcattgttggtctgcctggtcagcgtggtgagagaggattcccaggccttcccggcccatcgggtgagcccggcaagcagggtgcacctggtgcatctggagacagaggtcctcctggtcctgtggggcctcctggcttgacaggacctgcaggtgaacctggacgagagggcagccctggtgctgatggaccccctggcagagatggtgcggctggagtcaagggtgatcgtggtgagactggtgcacttggtgctcctggagctcctgggcccccaggctctcctggtcctgctggcccaactggcaaacaaggagacagaggagaggctggtgcacaaggtcctatgggcccctcaggacctgctggagcccgtggaattgctggccctcaaggcccccgaggtgacaaaggagaagctggagagcctggcgagagaggactgaaggggcaccgaggtttcactggactgcagggtctgcctggccccccgggtccttctggagatcagggtacttctggccctgctggtccttccggccctagaggtccacctggccctgttggtccctctggcaaagatggctctaatggaatccctggccccatcgggcctccaggtccccgtggacgctcaggagaaactggccctgctggtcctcctggaaatcctggtccccctggccctccgggtcctcctggtcctggcatcgacatgtcagcctttgctggcttaggacagagagagaagggccccgatcccctgcagtacatgcgggccgacgaggcagacagtaccttgagacagcatgacgtcgaggtggacgccacgctcaagtcgctgaacaaccagatcgagagcatccgcagccctgatggctcccgcaagaatcccgctcgcacctgccaggacctgaaactctgccacccagagtggaagagcggagactactggattgatcccaaccagggctgcaccttggacgccatgaaagtcttctgcaacatggagactggcgagtcttgcgtctaccccaacccagcgactgtgcctcggaagaactggtggagcagcaagagcaaggagaagaagcacatctggtttggagagaccatgaacggcggcttccacttcagctacggcgacggcaacctggctcccaacaccgctaacgtccagatgactttcctccgtctactgtccactgagggctcccagaacatcacctaccactgtaagaacagcattgcctacctggacgaagcagccggcaacctcaagaaggccttgctcatccagggctccaatgatgtggagatgagggccgagggcaacagcaggttcacgtacactgccctgaaggatggctgcacgaaacacaccggtaagtggggcaagaccatcatcgagtaccgatcacagaagacctcacgccttcccattgttgacattgcacccatggacatcggagggcctgatcaggaatttggtgtggacatagggcctgtctgtttcttgtaaaaccctcaaccccaaaacaacacaatccattgcgaacccaaaggacccaaatactttctaaccgcagtcactctaggatctgcactgaatggctgacctgacctgatattcaactatcctaacctcacagtccggac

SEQ ID NO: 3 - DNA, 4530 bp, Rattus norvegicus
  source 1..4530: mol_type = genomic DNA
ggctgccgggtctcctgcctcctcctcctgctcctagagcctcctgcatgagggagacccggacccgctccgtgctctgccgcctcgccgagcttcgcccgggccaaggctctgccaggcctcgcggtgagccatgatccgcctcggggctccccagtcgctggtgctgctgacgctgctcatcgccacggtcctacaatgtcagggccaggatgcccgaaaattagggccaaaggggcagaaaggagaacctggagatatcaaagatatcataggacctaaaggacctcctggccctcagggacctgccggtgaacaaggacccagaggtgaccgtggtgacaagggagagaggggtgcacctggaccccgtggcagagatggagaacctggtacccctggaaatcctggtccccctggccctccaggcccccctggtccccctggccttggtggaggaaactttgcagcccagatggctggaggatttgacgagaaggctggtggtgcccagatgggagtcatgcaaggccccatgggccccatgggacctcgtggacccccaggccccgccggtgcccccggccctcaaggatttcaaggcaatcctggtgaacctggcgagcctggtgtctctggtcccattggtccccgaggtcctccaggtcctgctggaaaacctggtgatgatggtgaagctggaaagcccggaaaggccggagaaagaggcctccctggtcctcagggtgctcgtggattcccgggaacccccggtcttcctggtgtcaagggtcacagaggttacccaggcctcgatggtgctaagggagaagctggtgctccaggtgtgaagggtgagagcggttcccctggtgagaacggatccccaggcccaatgggtccccgtggcctgcctggcgagagaggacggactggccctgctggtgctgctggtgctcgaggcaacgacggccagccaggccctgctggacctccgggtcctgttggtcctgcaggtggtcctggcttccttggtgctcctggtgccaagggcgaagctggtcccactggtgcccgtggtcctgaaggtgctcaaggttctcgtggcgaacccggcaatcccggatcccccgggcccgcaggcgcttctggtaacccagggactgatggtattcccggagccaaaggatctgctggcgctcctggaattgctggtgcccctggcttccctgggccccgtggccctcccggtcctcaaggtgcaactggtcctctgggccccaaaggtcagacgggtgagcccggcatcgctggcttcaaaggtgaacaaggccccaagggagagactggacctgctgggccccagggagcccctggccctgctggtgaagaaggaaaacgaggtgctcgaggagagcccggtggcgctggacctatcggcccccctggagagagaggtgctcctggcaaccgcggtttcccaggtcaagatggtctggcaggtcccaagggtgcccctggagagcgagggcctagtggcctggctggtcctaagggtgccaatggtgacccgggtcgtcctggagaacctggtcttcctggagccaggggtcttactggccgccctggtgatgctggtcctcaaggcaaagttggtccttctggagcccctggagaagacggtcgccctggtcctcctggtcctcagggagctcgtgggcagcctggcgtcatgggtttccctggccccaaaggagccaatggcgagcctggcaaagctggtgagaaaggactggctggtgctcctggtctgagaggtcttcctggcaaagatggtgagacaggagccgcaggaccccccggccccagcggacctgctggtgaacgaggcgagcagggtgctcctgggccatcagggttccagggacttcctggccctcctggtcccccgggtgaaggtggaaagcaaggtgaccagggtattcctggtgaagctggagcccctggcctcgttggtccccggggtgaacgaggtttcccaggtgaacgtggctctcccggtgctcagggcctccagggtccccgaggcctccctggcactcctggtactgatggtcccaaaggtgcggctggcccagatggtccccctggggctcagggccctccaggtctacagggaatgcctggtgagaggggagcagctggtattgctggacccaagggagacagaggtgatgttggcgagaaaggcccagagggagctcctggaaaagatggtggccgaggtcttactgggcccatcgggcccccaggaccagcaggtgccaatggcgagaagggagaagtcggacctcctggtccttcaggaagtactggagctcgaggcgccccgggtgagcgcggagagactgggccacctggacctgctggattcgctggccctcctggtgctgatggccagcctggtgccaagggcgatcaaggagaagctggacagaaaggtgacgctggtgcccctggcccacaaggcccctcaggagctcccgggccacagggtcctactggagtgactggtcctaagggagcccggggcgcccaaggcccaccgggagccaccggattccctggagctgctggccgagttggacccccaggttctaatggcaaccctgggcccgccggtccccctggtcctgctggaaaagatggtcccaaaggtgctcgaggagacactggtgcccctggcagagctggtgaccctggacttcaaggacccgcaggagctcctggagagaaaggcgaacctggagatgacggtccctctggttctgatggtcccccaggtccccaggggctggctggtcaaaggggcattgttggtctgcctggtcagcgtggtgagagaggattcccaggccttcccggcccatcgggtgagcccggcaagcagggtgcacctggtgcatctggagacagaggtcctcctggtcctgtggggcctcctggcttgacaggacctgcaggtgaacctggacgagagggcagccctggtgctgatggaccccctggcagagatggtgcggctggagtcaagggtgatcgtggtgagactggtgcacttggtgctcctggagctcctgggcccccaggctctcctggtcctgctggcccaactggcaaacaaggagacagaggagaggctggtgcacaaggtcctatgggcccctcaggacctgctggagcccgtggaattgctggccctcaaggcccccgaggtgacaaaggagaagctggagagcctggcgagagaggactgaaggggcaccgaggtttcactggactgcagggtctgcctggccccccgggtccttctggagatcagggtacttctggccctgctggtccttccggccctagaggtccacctggccctgttggtccctctggcaaagatggctctaatggaatccctggccccatcgggcctccaggtccccgtggacgctcaggagaaactggccctgctggtcctcctggaaatcctggtccccctggccctccgggtcctcctggtcctggcatcgacatgtcagcctttgctggcttaggacagagagagaagggccccgatcccctgcagtacatgcgggccgacgaggcagacagtaccttgagacagcatgacgtcgaggtggacgccacgctcaagtcgctgaacaaccagatcgagagcatccgcagccctgatggctcccgcaagaatcccgctcgcacctgccaggacctgaaactctgccacccagagtggaagagcggagactactggattgatcccaaccagggctgcaccttggacgccatgaaagtcttctgcaacatggagactggcgagtcttgcgtctaccccaacccagcgactgtgcctcggaagaactggtggagcagcaagagcaaggagaagaagcacatctggtttggagagaccatgaacggcggcttccacttcagctacggcgacggcaacctggctcccaacaccgctaacgtccagatgactttcctccgtctactgtccactgagggctcccagaacatcacctaccactgtaagaacagcattgcctacctggacgaagcagccggcaacctcaagaaggccttgctcatccagggctccaatgatgtggagatgagggccgagggcaacagcaggttcacgtacactgccctgaaggatggctgcacgaaacacaccggtaagtggggcaagaccatcatcgagtaccgatcacagaagacctcacgccttcccattgttgacattgcacccatggacatcggagggcctgatcaggaatttggtgtggacatagggcctgtctgtttcttgtaaaaccctcaaccccaaaacaacacaatccattgcgaacccaaaggacccaaatactttctaaccgcagtcactctaggatctgcactgaatggctgacctgacctgatattcaactatcctaacctcacagtccggac

SEQ ID NO: 4 - protein, 1419 aa, Rattus norvegicus
MIRLGAPQSLVLLTLLIATVLQCQGQDARKLGPKGQKGEPGDIKDIIGPKGPPGPQGPAGEQGPRGDRGDKGERGAPGPRGRDGEPGTPGNPGPPGPPGPPGPPGLGGGNFAAQMAGGFDEKAGGAQMGVMQGPMGPMGPRGPPGPAGAPGPQGFQGNPGEPGEPGVSGPIGPRGPPGPAGKPGDDGEAGKPGKAGERGLPGPQGARGFPGTPGLPGVKGHRGYPGLDGAKGEAGAPGVKGESGSPGENGSPGPMGPRGLPGERGRTGPAGAAGARGNDGQPGPAGPPGPVGPAGGPGFLGAPGAKGEAGPTGARGPEGAQGSRGEPGNPGSPGPAGASGNPGTDGIPGAKGSAGAPGIAGAPGFPGPRGPPGPQGATGPLGPKGQTGEPGIAGFKGEQGPKGETGPAGPQGAPGPAGEEGKRGARGEPGGAGPIGPPGERGAPGNRGFPGQDGLAGPKGAPGERGPSGLAGPKGANGDPGRPGEPGLPGARGLTGRPGDAGPQGKVGPSGAPGEDGRPGPPGPQGARGQPGVMGFPGPKGANGEPGKAGEKGLAGAPGLRGLPGKDGETGAAGPPGPSGPAGERGEQGAPGPSGFQGLPGPPGPPGEGGKQGDQGIPGEAGAPGLVGPRGERGFPGERGSPGAQGLQGPRGLPGTPGTDGPKGAAGPDGPPGAQGPPGLQGMPGERGAAGIAGPKGDRGDVGEKGPEGAPGKDGGRGLTGPIGPPGPAGANGEKGEVGPPGPSGSTGARGAPGERGETGPPGPAGFAGPPGADGQPGAKGDQGEAGQKGDAGAPGPQGPSGAPGPQGPTGVTGPKGARGAQGPPGATGFPGAAGRVGPPGSNGNPGPAGPPGPAGKDGPKGARGDTGAPGRAGDPGLQGPAGAPGEKGEPGDDGPSGSDGPPGPQGLAGQRGIVGLPGQRGERGFPGLPGPSGEPGKQGAPGASGDRGPPGPVGPPGLTGPAGEPGREGSPGADGPPGRDGAAGVKGDRGETGALGAPGAPGPPGSPGPAGPTGKQGDRGEAGAQGPMGPSGPAGARGIAGPQGPRGDKGEAGEPGERGLKGHRGFTGLQGLPGPPGPSGDQGTSGPAGPSGPRGPPGPVGPSGKDGSNGIPGPIGPPGPRGRSGETGPAGPPGNPGPPGPPGPPGPGIDMSAFAGLGQREKGPDPLQYMRADEADSTLRQHDVEVDATLKSLNNQIESIRSPDGSRKNPARTCQDLKLCHPEWKSGDYWIDPNQGCTLDAMKVFCNMETGESCVYPNPATVPRKNWWSSKSKEKKHIWFGETMNGGFHFSYGDGNLAPNTANVQMTFLRLLSTEGSQNITYHCKNSIAYLDEAAGNLKKALLIQGSNDVEMRAEGNSRFTYTALKDGCTKHTGKWGKTIIEYRSQKTSRLPIVDIAPMDIGGPDQEFGVDIGPVCFL

SEQ ID NO: 5 - protein, 1464 aa, Rattus norvegicus
  SITE 29: note = misc_feature - X is stop codon
  SITE 45: note = misc_feature - X is stop codon
  SITE 237: note = misc_feature - X is stop codon
  SITE 558: note = misc_feature - X is stop codon
  SITE 810: note = misc_feature - X is stop codon
  SITE 957: note = misc_feature - X is stop codon
  SITE 1059: note = misc_feature - X is stop codon
  SITE 1156: note = misc_feature - X is stop codon
  SITE 1178: note = misc_feature - X is stop codon
  SITE 1192: note = misc_feature - X is stop codon
  SITE 1216: note = misc_feature - X is stop codon
  SITE 1241: note = misc_feature - X is stop codon
  SITE 1283: note = misc_feature - X is stop codon
  SITE 1305: note = misc_feature - X is stop codon
  SITE 1351: note = misc_feature - X is stop codon
  SITE 1364: note = misc_feature - X is stop codon
  SITE 1411: note = misc_feature - X is stop codon
  SITE 1438: note = misc_feature - X is stop codon
  SITE 1443: note = misc_feature - X is stop codon
  SITE 1447: note = misc_feature - X is stop codon
  SITE 1453: note = misc_feature - X is stop codon
  SITE 1464: note = misc_feature - X is stop codon
MIRLGAPQSLVLLTLLIAYNVRARMPENXGQRGRKENLEISKISXDLKDLLALRDLPVNKDPEVTVVTRERGVHLDPVAEMENLVPLEILVPLALQAPLVPLALVEETLQPRWLEDLTRRLVVPRWESCKAPWAPWDLVDPQAPPVPPALKDFKAILVNLASLVSLVPLVPEVLQVLLENLVMMVKLESPERPEKEASLVLRVLVDSREPPVFLVSRVTEVTQASMVLREKLVLQVXRVRAVPLVRTDPQAQWVPVACLAREDGLALLVLLVLEATTASQALLDLRVLLVLQVVLASLVLLVPRAKLVPLVPVVLKVLKVLVANPAIPDPPGPQALLVTQGLMVFPEPKDLLALLELLVPLASLGPVALPVLKVQLVLWAPKVRRVSPASLASKVNKAPRERLDLLGPREPLALLVKKENEVLEESPVALDLSAPLEREVLLATAVSQVKMVWQVPRVPLESEGLVAWLVLRVPMVTRVVLENLVFLEPGVLLAALVMLVLKAKLVLLEPLEKTVALVLLVLRELVGSLASWVSLAPKEPMASLAKLVRKDWLVLLVXEVFLAKMVRQEPQDPPAPADLLVNEASRVLLGHQGSRDFLALLVPRVKVESKVTRVFLVKLEPLASLVPGVNEVSQVNVALPVLRASRVPEASLALLVLMVPKVRLAQMVPLGLRALQVYRECLVRGEQLVLLDPRETEVMLARKAQRELLEKMVAEVLLGPSGPQDQQVPMARREKSDLLVLQEVLELEAPRVSAERLGHLDLLDSLALLVLMASLVPRAIKEKLDRKVTLVPLAHKAPQELPGHRVLLEXLVLREPGAPKAHREPPDSLELLAELDPQVLMATLGPPVPLVLLEKMVPKVLEETLVPLAELVTLDFKDPQELLERKANLEMTVPLVLMVPQVPRGWLVKGALLVCLVSVVREDSQAFPAHRVSPASRVHLVHLETEVLLVLWGLLAXQDLQVNLDERAALVLMDPLAEMVRLESRVIVVRLVHLVLLELLGPQALLVLLAQLANKETEERLVHKVLWAPQDLLEPVELLALKAPEVTKEKLESLAREDXRGTEVSLDCRVCLAPRVLLEIRVLLALLVLPALEVHLALLVPLAKMALMESLAPSGLQVPVDAQEKLALLVLLEILVPLALRVLLVLASTCQPLLAXDRERRAPIPCSTCGPTRQTVPXDSMTSRWTPRSSRXTTRSRASAALMAPARIPLAPARTXNSATQSGRAETTGLIPTRAAPWTPXKSSATWRLASLASTPTQRLCLGRTGGAARARRRSTSGLERPXTAASTSATATATWLPTPLTSRXLSSVYCPLRAPRTSPTTVRTALPTWTKQPATSRRPCSSRAPMMWRXGPRATAGSRTLPXRMAARNTPVSGARPSSSTDHRRPHAFPLLTLHPWTSEGLIRNLVWTXGLSVSCKTLNPKTTQSIANPKDPNTFXPQSLXDLHXMADLTXYSTILTSQSGX

SEQ ID NO: 6 - protein, 1466 aa, Rattus norvegicus
  SITE 20: note = misc_feature - X is Val, Ala, Asp or Gly
  SITE 50: note = misc_feature - X is stop codon
  SITE 61: note = misc_feature - X is stop codon
  SITE 67: note = misc_feature - X is stop codon
  SITE 70: note = misc_feature - X is stop codon
  SITE 120: note = misc_feature - X is stop codon
  SITE 161: note = misc_feature - X is stop codon
  REGION 185..186: note = misc_feature - X is stop codon
  SITE 188: note = misc_feature - X is stop codon
  SITE 231: note = misc_feature - X is stop codon
  SITE 242: note = misc_feature - X is stop codon
  SITE 248: note = misc_feature - X is stop codon
  SITE 318: note = misc_feature - X is stop codon
  SITE 341: note = misc_feature - X is stop codon
  SITE 345: note = misc_feature - X is stop codon
  SITE 389: note = misc_feature - X is stop codon
  SITE 398: note = misc_feature - X is stop codon
  SITE 419: note = misc_feature - X is stop codon
  SITE 468: note = misc_feature - X is stop codon
  SITE 474: note = misc_feature - X is stop codon
  SITE 479: note = misc_feature - X is stop codon
  SITE 500: note = misc_feature - X is stop codon
  SITE 551: note = misc_feature - X is stop codon
  SITE 569: note = misc_feature - X is stop codon
  SITE 584: note = misc_feature - X is stop codon
  SITE 608: note = misc_feature - X is stop codon
  SITE 614: note = misc_feature - X is stop codon
  SITE 620: note = misc_feature - X is stop codon
  SITE 632: note = misc_feature - X is stop codon
  SITE 638: note = misc_feature - X is stop codon
  SITE 660: note = misc_feature - X is stop codon
  SITE 686: note = misc_feature - X is stop codon
  SITE 701: note = misc_feature - X is stop codon
  SITE 755: note = misc_feature - X is stop codon
  SITE 774: note = misc_feature - X is stop codon
  SITE 791: note = misc_feature - X is stop codon
  SITE 816: note = misc_feature - X is stop codon
  SITE 843: note = misc_feature - X is stop codon
  SITE 875: note = misc_feature - X is stop codon
  SITE 894: note = misc_feature - X is stop codon
  SITE 900: note = misc_feature - X is stop codon
  SITE 923: note = misc_feature - X is stop codon
  SITE 935: note = misc_feature - X is stop codon
  SITE 965: note = misc_feature - X is stop codon
  SITE 975: note = misc_feature - X is stop codon
  SITE 989: note = misc_feature - X is stop codon
  SITE 992: note = misc_feature - X is stop codon
  SITE 1049: note = misc_feature - X is stop codon
  SITE 1095: note = misc_feature - X is stop codon
  SITE 1110: note = misc_feature - X is stop codon
  SITE 1184: note = misc_feature - X is stop codon
  SITE 1205: note = misc_feature - X is stop codon
  SITE 1233: note = misc_feature - X is stop codon
  SITE 1304: note = misc_feature - X is stop codon
  SITE 1316: note = misc_feature - X is stop codon
  SITE 1326: note = misc_feature - X is stop codon
  SITE 1350: note = misc_feature - X is stop codon
  SITE 1376: note = misc_feature - X is stop codon
  SITE 1396: note = misc_feature - X is stop codon
  SITE 1406: note = misc_feature - X is stop codon
  SITE 1454: note = misc_feature - X is stop codon
  SITE 1461: note = misc_feature - X is stop codon
MIRLGAPQSLVLLTLLIATXPTMSGPGCPKIRAKGAERRTWRYQRYHRTXRTSWPSGTCRXTRTQRXPWXQGREGCTWTPWQRWRTWYPWKSWSPWPSRPPWSPWPWWRKLCSPDGWRIXREGWWCPDGSHARPHGPHGTSWTPRPRRCPRPSRISRQSWXTWRAWCLWSHWSPRSSRSCWKTWXXWXSWKARKGRRKRPPWSSGCSWIPGNPRSSWCQGSQRLPRPRWCXGRSWCSRCEGXERFPWXERIPRPNGSPWPAWRERTDWPCWCCWCSRQRRPARPCWTSGSCWSCRWSWLPWCSWCQGRSWSHWCPWSXRCSRFSWRTRQSRIPRARRRFWXPRDXWYSRSQRICWRSWNCWCPWLPWAPWPSRSSRCNWSSGPQRSDGXARHRWLQRXTRPQGRDWTCWAPGSPWPCWXRRKTRCSRRARWRWTYRPPWRERCSWQPRFPRSRWSGRSQGCPWRARAXWPGWSXGCQWXPGSSWRTWSSWSQGSYWPPWXCWSSRQSWSFWSPWRRRSPWSSWSSGSSWAAWRHGFPWPQRSQWRAWQSWXERTGWCSWSERSSWQRWXDRSRRTPRPQRTCWXTRRAGCSWAIRVPGTSWPSWSPGXRWKARXPGYSWXSWSPWPRWSPGXTRFPRXTWLSRCSGPPGSPRPPWHSWYXWSQRCGWPRWSPWGSGPSRSTGNAWXEGSSWYCWTQGRQRXCWRERPRGSSWKRWWPRSYWAHRAPRTSRCQWREGRSRTSWSFRKYWSSRRPGXARRDWATWTCWIRWPSWCXWPAWCQGRSRRSWTERXRWCPWPTRPLRSSRATGSYWSDWSXGSPGRPRPTGSHRIPWSCWPSWTPRFXWQPWARRSPWSCWKRWSQRCSRRHWCPWQSWXPWTSRTRRSSWRERRTWRXRSLWFXWSPRSPGAGWSKGHCWSAWSAWXERIPRPSRPIGXARQAGCTWCIWRQRSSWSCGASWLDRTCRXTWTRGQPWCXWTPWQRWCGWSQGXSWXDWCTWCSWSSWAPRLSWSCWPNWQTRRQRRGWCTRSYGPLRTCWSPWNCWPSRPPRXQRRSWRAWRERTEGAPRFHWTAGSAWPPGSFWRSGYFWPCWSFRPXRSTWPCWSLWQRWLXWNPWPHRASRSPWTLRRNWPCWSSWKSWSPWPSGSSWSWHRHVSLCWLRTEREGPRSPAVHAGRRGRQYLETAXRRGGRHAQVAEQPDREHPQPXWLPQESRSHLPGPETLPPRVEERRLLDXSQPGLHLGRHESLLQHGDWRVLRLPQPSDCASEELVEQQEQGEEAHLVWRDHERRLPLQLRRRQPGSQHRXRPDDFPPSTVHXGLPEHHLPLXEQHCLPGRSSRQPQEGLAHPGLQXCGDEGRGQQQVHVHCPEGWLHETHRXVGQDHHRVPITEDLTPSHCXHCTHGHRRAXSGIWCGHRACLFLVKPSTPKQHNPLRTQRTQILSNRSHSRICTEWLTXPDIQLSXPHSPD

SEQ ID NO: 7 - DNA, 2115 bp, Rattus norvegicus
  source 1..2115: mol_type = genomic DNA
ttttctccgagttttctgaactctggctcatgatcgggcttactggatacgagatcctggaggaccgtaccctgatctccatctacctctgactttgagcctttctaacccggggctcacgctgccaacacccgggccacctggtccgatcgtcttacttcattcaccagcgttgccaattgctgccctgtccccagccccaatgggggagtgagagaggccactgccggccggacatgggtctccccatcgtgcctggcctgctgctgtcactggtgctcctggctctgctgatggggatacacccgtcaggggtcaccggactggttccttctcttggtgaccgggagaagagggataatttgtgtccccagggaaagtatgcccatccaaagaataattccatctgctgcaccaagtgccacaaaggaacctacttggtgagtgactgtccaagcccagggcaggaaacagtctgcgaggtgtgtgataaaggcacctttacagcttcgcagaaccacgtcagacagtgtctcagttgcaagacatgtcggaaagaaatgttccaggtggagatttctccttgcaaagctgacatggacaccgtgtgtggctgcaagaagaaccaattccagcgctacctgagtgagacgcatttccagtgtgtggactgcagcccctgcttcaatggcaccgtgacaatcccctgtaaggagaaacagaacaccgtgtgtaactgccacgcaggattctttctaagcggaaatgagtgcaccccttgcagccactgcaagaaaaatcaggaatgtatgaagctgtgcctacctccagttgcaaatgtcacaaacccccaggactcaggtactgccgtgctgttgcctctggttatcttcctaggtctttgccttttattctttatctgcatcagtctactgtgccgatatccccagtggaggcccagggtctactccatcatttgtagggattcagctcctgtcaaagaggtggagggtgaaggaattgttactaagcccctaactccagcctctatcccagccttcagccccaaccccggcttcaaccccactctgggcttcagcaccaccccacgcttcagtcctcctgtctccagtacccccatcagccccgtcttcggtcctagtaactggcacaacttcgtgccacctgtaagagaggtggtcccaacccagggtgctgaccctctcctctacggatccctcaaccctgtgccaatccccgcccctgttcggaaatgggaagacgtcgtcgcggcccagccacaacggcttgacactgcagaccctgcgatgctgtatgctgtggtggatggcgtgcctccgacacgctggaaggagttcatgcggctcctggggctgagcgagcacgagatcgagcggctggagctgcagaacgggcgttgcctccgcgaggctcattacagcatgctggaagcctggcggcgccgcacaccgcgacacgaggccacgctggacgtagtgggccgcgtgctttgcgacatgaacctgcgtggctgcctggagaacatccgcgagactctagaaagccctgcccactcgtccacgacccacctcccgcgataaggccacacccccacctcaggaacgggactcgaaggaccatcctgctagatgccctgcttccctgtgaacctcctctttggtcctctagggggcaggctcgatctggcagccacttccttggtgctaccgacttggtgtacatagcttttcccagctgccgaggacagcctgtgccagccacttgtgcatggcagggaagtgtgccatctgctcccagacagctgagggtgccaaaagccaggagaggtgattgtggagaaaaagcacaatctatctgatacccacttgggatgcaaggacccaaacaaagcttctcagggcctcctcagttgatttctgggcccttttcacagtagataaaacagtctttgtattgattatatcacactaatggatgaacggttgaactccctaaggtaggggcaagcacagaacagtggggtctccagctggagcccccgactcttgtaaatacactaaaaatctaaaagtg

SEQ ID NO: 8 - protein, 461 aa, Rattus norvegicus
MGLPIVPGLLLSLVLLALLMGIHPSGVTGLVPSLGDREKRDNLCPQGKYAHPKNNSICCTKCHKGTYLVSDCPSPGQETVCEVCDKGTFTASQNHVRQCLSCKTCRKEMFQVEISPCKADMDTVCGCKKNQFQRYLSETHFQCVDCSPCFNGTVTIPCKEKQNTVCNCHAGFFLSGNECTPCSHCKKNQECMKLCLPPVANVTNPQDSGTAVLLPLVIFLGLCLLFFICISLLCRYPQWRPRVYSIICRDSAPVKEVEGEGIVTKPLTPASIPAFSPNPGFNPTLGFSTTPRFSHPVSSTPISPVFGPSNWHNFVPPVREVVPTQGADPLLYGSLNPVPIPAPVRKWEDVVAAQPQRLDTADPAMLYAVVDGVPPTRWKEFMRLLGLSEHEIERLELQNGRCLREAHYSMLEAWRRRTPRHEATLDVVGRVLCDMNLRGCLENIRETLESPAHSSTTHLPR

SEQ ID NO: 9 - protein, 462 aa, Rattus norvegicus
  SITE 19: note = misc_feature - X is stop codon
  SITE 69: note = misc_feature - X is stop codon
  SITE 136: note = misc_feature - X is stop codon
  SITE 154: note = misc_feature - X is stop codon
  SITE 174: note = misc_feature - X is stop codon
  SITE 192: note = misc_feature - X is stop codon
  SITE 220: note = misc_feature - X is stop codon
  SITE 267: note = misc_feature - X is stop codon
  SITE 318: note = misc_feature - X is stop codon
  SITE 387: note = misc_feature - X is stop codon
  SITE 427: note = misc_feature - X is stop codon
  SITE 435: note = misc_feature - X is stop codon
  SITE 448: note = misc_feature - X is stop codon
  SITE 462: note = misc_feature - X is stop codon
MGLPICLACCCHWCSWLCXWGYTHQGSPDWFLLLVTGRRGIICVPRESMPIQRIIPSAAPSATKEPTWXVTVQAQGRKQSARCVIKAPLQLRRTTSDSVSVARHVGKKCSRWRFLLAKLTWTPCVAARRTNSSATXVRRISSVWTAAPASMAPXQSPVRRNRTPCVTATQDSFXAEMSAPLAATARKIRNVXSCAYLQLQMSQTPRTQVLPCCCLWLSSXVFAFYSLSASVYCADIPSGGPGSTPSFVGIQLLSKRWRVKELLLSPXLQPLSQPSAPTPASTPLWASAPPHASVILSPVPPSAPSSVLVTGTTSCHLXERWSQPRVLTLSSTDPSTLCQSPPLFGNGKTSSRPSHNGLTLQTLRCCMLWWMACLRHAGRSSCGSWGXASTRSSGWSCRTGVASARLITACWKPGGAAHRDTRPRWTXWAACFATXTCVAAWRTSARLXKALPTRPRPTSRDX

SEQ ID NO: 10 - DNA, 3005 bp, Rattus norvegicus
  source 1..3005: mol_type = genomic DNA
cttttcccagacactttcacgtggggcacaaagaaggctttgaagcagagacttgaaatgcctgtgaagatggtcgcgatcttcggagcctcaacggtactttggatactgtttgcagtctctcaagcttttaaaatcgagatctcccctgaatacaaaacgctcgctcagattggagactccatgctcctgacttgcagcaccacaggctgtgagtcgccatcattctcttggagaacccagatagacagtccactaaatgggaaggtgaagacagagggggccaagtccgttctgaccatggaccctgtcagctttgagaatgaacactcttacctgtgcacagcaacatgtaactctgggaaactggaaagaggaatccaagtggacatctactcattccctaaggatccagagattcaattcagtggccccctggaggttgggaagccggtcatggtcaagtgtttggctcctgatgtttacccaattgacagactggagatagaactgttcaagggtgaccgtctcatgaagaaacaggattttgtagacgagatggcaaagaagtctctggaaaccaagagtttggaagtcatctttactcctgtcattgaggatattgaaaaggctcttgtttgccgagctaaattatacattgaccaaactgattctattcccaaagaaagggagactgtcagagaactacaagtctacacctcccccaagaatacagagatctctgtacatccctccacaaggctacatgagggtgctgctgtgacgatgacatgtgccagcgagggtctaccagctcctgagattttctggagcaagaaattagataatggagttctacagctcctctcgggaaatgccaccctcaccttaattgctatgaggatggaagattctggaatctatgtgtgtgaaggagtgaatctggttgggagagacaaaacagaagtggaattaattgttcaagagaaaccatttactgttgacatctcccctggatctcaggtggctgcacaggttggggattccgttgttctgacatgtgctgctgttggctgtgactctccctccttttcttggagaacccagacagacagtcccctcaatggggaggtgagggatgaaggggctacatccacactgacgctgagccctgtgggtgttgaggatgagcactcttacctgtgcactgtgacctgtcagcgaaggaaactggagaagacaatccaagtggaggtctactcattccctgaagacccagaaattgaaataagtggaccacttgtacacgggagacctgtcactgtcaactgcacggtccctaatgtgtacccctttgaccatctggagattgaactactgaagggggagacaacactgttgaataaatttttaagggaggaaattggcacaaagtctctagagaccaaaagtttggaaatgaccttcatccccaccgctgaagacaccgggaaagctcttgtttgcctcgctaagttacacagcagtcaaatggagtctgaacccaaacaaaggcagagtacacagactctttatgtcaacgttgctccgaaagaacccaccatctgggttagcccctctcctgtcccagaggagggcagtcctgtgaacctgacctgctcaagtgatggttttccaactcccaaaatcctgtggagcagacagctaaagaacggggaactgcagcctctttctcaaaatacaacactctccttcatggctacaaaaatggaagattccggcatttatgtatgtgaagggattaatgaggctggaattagcaaaaaatcagttgaactgattatccaaggctcttcgaaggacatacagcttacagtcttcccatctaagagcgtcaaagagggagacactgtcattatctcctgtacttgtggaagtgtgcccgaaatatggataattctgaaaaagaaagccaagacaggagacatggtgctaaagtctgttaatggctcgtacaccatccgcaaggcacagctgcaggatgccggagtatacgagtgtgaatcgaaaaccgaagtcggctcgcagttgcgaagtttaacacttgatgtgaaaggaaaagaaaataacaaggactatttttcccctgaactccttgcactctactttgcatcctccttggtaatacccgccattgggatgatcatttactttgcaagaaaagccaacatgaaaggatcgtacagtctggtggaggcacagaagtcaaaagtgtagctaacgtctgaactgttggagaaaagacattatttataaaccccggacccttcatactctttattgcagcactgttccccctccacaaaccaagctatgcattcagacttctcagaacccttctcggcaaagaaggaaaagaagtggccacttgatcccttgctgagtgcaagaagccaactagaaatcttctgctcggcaagtccccattgctgaagagaccggaacagtaccatgacatgtatataaatagcctcagtgtacatatgtaaaataaaatgatgtcattgcgaggtcgtttagagtagtagcactccagatgtaggtcagaacaaaatcaaaacgtgttgcttggactgactgttgtaacttcatgcttcttaggaaagtttaatgttggtgttaatgttgagtaggcagctgaccagtgtcacctttttgtactttattttcttcagcctaattttattcctatgcattttattgacaatgatttcatttttttttaaagaagccagggttttatatttttataggcaaatggtaaaaaggtcactgggttgactttcaggtactactttcctaattcatggtatactgattaagtagttttctcaactgtacggtacggggacgtgtttcttcatcaggatcttgtataatgactaacatggtttaaatgcaacttcatttgacttataaatactacagtaaagtgaaagtttctg

SEQ ID NO: 11 - protein, 739 aa, Rattus norvegicus
MPVKMVAIFGASTVLWILFAVSQAFKIEISPEYKTLAQIGDSMLLTCSTTGCESPSFSWRTQIDSPLNGKVKTEGAKSVLTMDPVSFENEHSYLCTATCNSGKLERGIQVDIYSFPKDPEIQFSGPLEVGKPVMVKCLAPDVYPIDRLEIELFKGDRLMKKQDFVDEMAKKSLETKSLEVIFTPVIEDIEKALVCRAKLYIDQTDSIPKERETVRELQVYTSPKNTEISVHPSTRLHEGAAVTMTCASEGLPAPEIFWSKKLDNGVLQLLSGNATLTLIAMRMEDSGIYVCEGVNLVGRDKTEVELIVQEKPFTVDISPGSQVAAQVGDSVVLTCAAVGCDSPSFSWRTQTDSPLNGEVRDEGATSTLTLSPVGVEDEHSYLCTVTCQRRKLEKTIQVEVYSFPEDPEIEISGPLVHGRPVTVNCTVPNVYPFDHLEIELLKGETTLLNKFLREEIGTKSLETKSLEMTFIPTAEDTGKALVCLAKLHSSQMESEPKQRQSTQTLYVNVAPKEPTIWVSPSPVPEEGSPVNLTCSSDGFPTPKILWSRQLKNGELQPLSQNTTLSFMATKMEDSGIYVCEGINEAGISKKSVELIIQGSSKDIQLTVFPSKSVKEGDTVIISCTCGSVPEIWIILKKKAKTGDMVLKSVNGSYTIRKAQLQDAGVYECESKTEVGSQLRSLTLDVKGKENNKDYFSPELLALYFASSLVIPAIGMIIYFARKANMKGSYSLVEAQKSKV

SEQ ID NO: 12 - protein, 739 aa, Rattus norvegicus
  SITE 356: note = misc_feature - X is stop codon
  SITE 370: note = misc_feature - X is stop codon
  SITE 372: note = misc_feature - X is stop codon
  SITE 399: note = misc_feature - X is stop codon
  SITE 404: note = misc_feature - X is stop codon
  SITE 423: note = misc_feature - X is stop codon
  SITE 428: note = misc_feature - X is stop codon
  SITE 433: note = misc_feature - X is stop codon
  SITE 444: note = misc_feature - X is stop codon
  SITE 469: note = misc_feature - X is stop codon
  SITE 480: note = misc_feature - X is stop codon
  SITE 489: note = misc_feature - X is stop codon
  SITE 513: note = misc_feature - X is stop codon
  SITE 531: note = misc_feature - X is stop codon
  SITE 574: note = misc_feature - X is stop codon
  REGION 577..578: note = misc_feature - X is stop codon
  SITE 582: note = misc_feature - X is stop codon
  SITE 587: note = misc_feature - X is stop codon
  SITE 605: note = misc_feature - X is stop codon
  SITE 644: note = misc_feature - X is stop codon
  SITE 663: note = misc_feature - X is stop codon
  SITE 678: note = misc_feature - X is stop codon
  SITE 685: note = misc_feature - X is stop codon
  SITE 692: note = misc_feature - X is stop codon
  SITE 738: note = misc_feature - X is stop codon
MPVKMVAIFGASTVLWILFAVSQAFKIEISPEYKTLAQIGDSMLLTCSTTGCESPSFSWRTQIDSPLNGKVKTEGAKSVLTMDPVSFENEHSYLCTATCNSGKLERGIQVDIYSFPKDPEIQFSGPLEVGKPVMVKCLAPDVYPIDRLEIELFKGDRLMKKQDFVDEMAKKSLETKSLEVIFTPVIEDIEKALVCRAKLYIDQTDSIPKERETVRELQVYTSPKNTEISVHPSTRLHEGAAVTMTCASEGLPAPEIFWSKKLDNGVLQLLSGNATLTLIAMRMEDSGIYVCEGVNLVGRDKTEVELIVQEKPFTVDISPGSQVAAQVGDSVVLTCAAVGCDSPSFSWRTQTDSEGXRGYIHTDAEPCGCXGXALLPVHCDLSAKETGEDNPSGGLLIPXRPRNXNKWTTCTRETCHCQLHGPXCVPLXPSGDXTTEGGDNTVEXIFKGGNWHKVSRDQKFGNDLHPHRXRHRESSCLPRXVTQQSNGVXTQTKAEYTDSLCQRCSERTHHLGXPLSCPRGGQSCEPDLLKXWFSNSQNPVEQTAKERGTAASFSKYNTLLHGYKNGRFRHLCMXRDXXGWNXQKISXTDYPRLFEGHTAYSLPIXERQRGRHCHYLLYLWKCARNMDNSEKESQDRRHGAKVCXWLVHHPQGTAAGCRSIRVXIENRSRLAVAKFNTXCERKRKXQGLFFPXTPCTLLCILLGNTRHWDDHLLCKKSQHERIVQSGGGTEVKSVANVXT